European Patent Specification EP 3 157 543 B1, published November 12, 2025. Title: COMPOSITIONS AND METHODS FOR THE DIAGNOSIS OF SYSTEMIC AUTOIMMUNE DISEASE. Applicant: INOVA DIAGNOSTICS, INC. The sequence listing filed with the application follows.

SEQUENCE LISTING (113 sequences)

SEQ ID NO: 1 - protein, 199 aa, Homo sapiens
MENFRKVRSEEAPAGCGAEGGGPGSGPFADLAPGAVHMRVKEGSKIRNLMAFATASMAQPATRAIVFSGCGRATTKTVTCAEILKRRLAGLHQVTRLRYRSVREVWQSLPPGPTQGQTPGEPAASLSVLKNVPGLAILLSKDALDPRQPGYQPPNPHPGPSSPPAAPASKRSLGEPAAGEGSAKRSQPEPGVADEDQTA

SEQ ID NO: 2 - protein, 283 aa, Homo sapiens
MAAAPQAPGRGSLRKTRPLVVKTSLNNPYIIRWSALESEDMHFILQTLEDRLKAIGLQKIEDKKKKNKTPFLKKESREKCSIAVDISENLKEKKTDAKQQVSGWTPAHVRKQLAIGVNEVTRALERRELLLVLVCKSVKPAMITSHLIQLSLSRSVPACQVPRLSERIAPVIGLKCVLALAFKKNTTDFVDEVRAIIPRVPSLSVPWLQDRIEDSGENLETEPLESQDRELLDTSFEDLSKPKRKLADGRQASVTLQPLKIKKLIPNPNKIRKPPKSKKATPK

SEQ ID NO: 3 - protein, 1024 aa, Homo sapiens
MSNAKERKHAKKMRNQPTNVTLSSGFVADRGVKHHSGGEKPFQAQKQEPHPGTSRQRQTRVNPHSLPDPEVNEQSSSKGMFRKKGGWKAGPEGTSQEIPKYITASTFAQARAAEISAMLKAVTQKSSNSLVFQTLPRHMRRRAMSHNVKRLPRRLQEIAQKEAEKAVHQKKEHSKNKCHKARRCHMNRTLEFNRRQKKNIWLETHIWHAKRFHMVKKWGYCLGERPTVKSHRACYRAMTNRCLLQDLSYYCCLELKGKEEEILKALSGMCNIDTGLTFAAVHCLSGKRQGSLVLYRVNKYPREMLGPVTFIWKSQRTPGDPSESRQLWIWLHPTLKQDILEEIKAACQCVEPIKSAVCIADPLPTPSQEKSQTELPDEKIGKKRKRKDDGENAKPIKKIIGDGTRDPCLPYSWISPTTGIIISDLTMEMNRFRLIGPLSHSILTEAIKAASVHTVGEDTEETPHRWWIETCKKPDSVSLHCRQEAIFELLGGITSPAEIPAGTILGLTVGDPRINLPQKKSKALPNPEKCQDNEKVRQLLLEGVPVECTHSFIWNQDICKSVTENKISDQDLNRMRSELLVPGSQLILGPHESKIPILLIQQPGKVTGEDRLGWGSGWDVLLPKGWGMAFWIPFIYRGVRVGGLKESAVHSQYKRSPNVPGDFPDCPAGMLFAEEQAKNLLEKYKRRPPAKRPNYVKLGTLAPFCCPWEQLTQDWESRVQAYEEPSVASSPNGKESDLRRSEVPCAPMPKKTHQPSDEVGTSIEHPREAEEVMDAGCQESAGPERITDQEASENHVAATGSHLCVLRSRKLLKQLSAWCGPSSEDSRGGRRAPGRGQQGLTREACLSILGHFPRALVWVSLSLLSKGSPEPHTMICVPAKEDFLQLHEDWHYCGPQESKHSDPFRSKILKQKEKKKREKRQKPGRASSDGPAGEEPVAGQEALTLGLWSGPLPRVTLHCSRTLLGFVTQGDFSMAVGCGEALGFVSLTGLLDMLSSQPAAQRGLVLLRPPASLQYRFARIAIEV

SEQ ID NO: 4 - protein, 15 aa, Homo sapiens
ATASMAQPATRAIVF

SEQ ID NO: 5 - protein, 15 aa, Homo sapiens
TASMAQPATRAIVFS

SEQ ID NO: 6 - protein, 15 aa, Homo sapiens
TQGQTPGEPAASLSV

SEQ ID NO: 7 - protein, 15 aa, Homo sapiens
EPAASLSVLKNVPGL

SEQ ID NO: 8 - protein, 15 aa, Homo sapiens
VPGLAILLSKDALDP

SEQ ID NO: 9 - protein, 15 aa, Homo sapiens
PGLAILLSKDALDPR

SEQ ID NO: 10 - protein, 15 aa, Homo sapiens
GLAILLSKDALDPRQ

SEQ ID NO: 11 - protein, 15 aa, Homo sapiens
AILLSKDALDPRQPG

SEQ ID NO: 12 - protein, 15 aa, Homo sapiens
LLSKDALDPRQPGYQ

SEQ ID NO: 13 - protein, 15 aa, Homo sapiens
KDALDPRQPGYQPPN

SEQ ID NO: 14 - protein, 15 aa, Homo sapiens
EPGVADEDQTAGSGS

SEQ ID NO: 15 - protein, 15 aa, Homo sapiens
GPGSGPFADLAPGAV

SEQ ID NO: 16 - protein, 15 aa, Homo sapiens
AFATASMAQPATRAI

SEQ ID NO: 17 - protein, 15 aa, Homo sapiens
FATASMAQPATRAIV

SEQ ID NO: 18 - protein, 15 aa, Homo sapiens
PTQGQTPGEPAASLS

SEQ ID NO: 19 - protein, 15 aa, Homo sapiens
AASLSVLKNVPGLAI

SEQ ID NO: 20 - protein, 15 aa, Homo sapiens
KNVPGLAILLSKDAL

SEQ ID NO: 21 - protein, 15 aa, Homo sapiens
RQPGYQPPNPHPGPS

SEQ ID NO: 22 - protein, 15 aa, Homo sapiens
SQDRELLDTSFEDLS

SEQ ID NO: 23 - protein, 15 aa, Homo sapiens
QDRELLDTSFEDLSK

SEQ ID NO: 24 - protein, 15 aa, Homo sapiens
DRELLDTSFEDLSKP

SEQ ID NO: 25 - protein, 15 aa, Homo sapiens
RELLDTSFEDLSKPK

SEQ ID NO: 26 - protein, 15 aa, Homo sapiens
ELLDTSFEDLSKPKR

SEQ ID NO: 27 - protein, 15 aa, Homo sapiens
LLDTSFEDLSKPKRK

SEQ ID NO: 28 - protein, 15 aa, Homo sapiens
LDTSFEDLSKPKRKL

SEQ ID NO: 29 - protein, 15 aa, Homo sapiens
PYIIRWSALESEDMH

SEQ ID NO: 30 - protein, 15 aa, Homo sapiens
SALESEDMHFILQTL

SEQ ID NO: 31 - protein, 15 aa, Homo sapiens
ESEDMHFILQTLEDR

SEQ ID NO: 32 - protein, 15 aa, Homo sapiens
TDAKQQVSGWTPAHV

SEQ ID NO: 33 - protein, 15 aa, Homo sapiens
PAHVRKQLAIGVNEV

SEQ ID NO: 34 - protein, 15 aa, Homo sapiens
AHVRKQLAIGVNEVT

SEQ ID NO: 35 - protein, 15 aa, Homo sapiens
KTSLNNPYIIRWSAL

SEQ ID NO: 36 - protein, 15 aa, Homo sapiens
MHFILQTLEDRLKAI

SEQ ID NO: 37 - protein, 15 aa, Homo sapiens
IEDKKKKNKTPFLKK

SEQ ID NO: 38 - protein, 15 aa, Homo sapiens
EDKKKKNKTPFLKKE

SEQ ID NO: 39 - protein, 15 aa, Homo sapiens
DKKKKNKTPFLKKES

SEQ ID NO: 40 - protein, 15 aa, Homo sapiens
KKKKNKTPFLKKESR

SEQ ID NO: 41 - protein, 15 aa, Homo sapiens
KKNKTPFLKKESREK

SEQ ID NO: 42 - protein, 15 aa, Homo sapiens
PFLKKESREKCSIAV

SEQ ID NO: 43 - protein, 15 aa, Homo sapiens
ISENLKEKKTDAKQQ

SEQ ID NO: 44 - protein, 15 aa, Homo sapiens
SENLKEKKTDAKQQV

SEQ ID NO: 45 - protein, 15 aa, Homo sapiens
ENLKEKKTDAKQQVS

SEQ ID NO: 46 - protein, 15 aa, Homo sapiens
KEKKTDAKQQVSGWT

SEQ ID NO: 47 - protein, 15 aa, Homo sapiens
KKTDAKQQVSGWTPA

SEQ ID NO: 48 - protein, 15 aa, Homo sapiens
VSGWTPAHVRKQLAI

SEQ ID NO: 49 - protein, 15 aa, Homo sapiens
RKQLAIGVNEVTRAL

SEQ ID NO: 50 - protein, 15 aa, Homo sapiens
ERIAPVIGLKCVLAL

SEQ ID NO: 51 - protein, 15 aa, Homo sapiens
RIAPVIGLKCVLALA

SEQ ID NO: 52 - protein, 15 aa, Homo sapiens
IAPVIGLKCVLALAF

SEQ ID NO: 53 - protein, 15 aa, Homo sapiens
FKKNTTDFVDEVRAI

SEQ ID NO: 54 - protein, 15 aa, Homo sapiens
DTSFEDLSKPKRKLA

SEQ ID NO: 55 - protein, 15 aa, Homo sapiens
TSFEDLSKPKRKLAD

SEQ ID NO: 56 - protein, 15 aa, Homo sapiens
SFEDLSKPKRKLADG

SEQ ID NO: 57 - protein, 15 aa, Homo sapiens
FEDLSKPKRKLADGR

SEQ ID NO: 58 - protein, 15 aa, Homo sapiens
KKLIPNPNKIRKPPK

SEQ ID NO: 59 - protein, 15 aa, Homo sapiens
KIRKPPKSKKATPKQ

SEQ ID NO: 60 - protein, 15 aa, Homo sapiens
ISDLTMEMNRFRLIG

SEQ ID NO: 61 - protein, 15 aa, Homo sapiens
GDPRINLPQKKSKAL

SEQ ID NO: 62 - protein, 15 aa, Homo sapiens
EISAMLKAVTQKSSN

SEQ ID NO: 63 - protein, 15 aa, Homo sapiens
ILKALSGMCNIDTGL

SEQ ID NO: 64 - protein, 15 aa, Homo sapiens
TGLTFAAVHCLSGKR

SEQ ID NO: 65 - protein, 15 aa, Homo sapiens
ADPLPTPSQEKSQTE

SEQ ID NO: 66 - protein, 15 aa, Homo sapiens
TRDPCLPYSWISPTT

SEQ ID NO: 67 - protein, 15 aa, Homo sapiens
TGIIISDLTMEMNRF

SEQ ID NO: 68 - protein, 15 aa, Homo sapiens
TMEMNRFRLIGPLSH

SEQ ID NO: 69 - protein, 15 aa, Homo sapiens
QLLLEGVPVECTHSF

SEQ ID NO: 70 - protein, 15 aa, Homo sapiens
EGVPVECTHSFIWNQ

SEQ ID NO: 71 - protein, 15 aa, Homo sapiens
KRSPNVPGDFPDCPA

SEQ ID NO: 72 - protein, 15 aa, Homo sapiens
EPHTMICVPAKEDFL

SEQ ID NO: 73 - protein, 15 aa, Homo sapiens
WHYCGPQESKHSDPF

SEQ ID NO: 74 - protein, 15 aa, Homo sapiens
GPQESKHSDPFRSKI

SEQ ID NO: 75 - protein, 15 aa, Homo sapiens
SDGPAGEEPVAGQEA

SEQ ID NO: 76 - protein, 15 aa, Homo sapiens
PVAGQEALTLGLWSG

SEQ ID NO: 77 - protein, 15 aa, Homo sapiens
TGLLDMLSSQPAAQR

SEQ ID NO: 78 - protein, 15 aa, Homo sapiens
ADRGVKHHSGGEKPF

SEQ ID NO: 79 - protein, 15 aa, Homo sapiens
NAKPIKKIIGDGTRD

SEQ ID NO: 80 - protein, 15 aa, Homo sapiens
REACLSILGHFPRAL

SEQ ID NO: 81 - protein, 16 aa, Homo sapiens
ATASMAQPATRAIVFS

SEQ ID NO: 82 - protein, 42 aa, Homo sapiens
TQGQTPGEPAASLSVLKNVPGLAILLSKDALDPRQPGYQPPN

SEQ ID NO: 83 - protein, 16 aa, Homo sapiens
AFATASMAQPATRAIV

SEQ ID NO: 84 - protein, 32 aa, Homo sapiens
PTQGQTPGEPAASLSVLKNVPGLAILLSKDAL

SEQ ID NO: 85 - protein, 21 aa, Homo sapiens
SQDRELLDTSFEDLSKPKRKL

SEQ ID NO: 86 - protein, 24 aa, Homo sapiens
PYIIRWSALESEDMHFILQTLEDR

SEQ ID NO: 87 - protein, 27 aa, Homo sapiens
TDAKQQVSGWTPAHVRKQLAIGVNEVT

SEQ ID NO: 88 - protein, 25 aa, Homo sapiens
IEDKKKKNKTPFLKKESREKCSIAV

SEQ ID NO: 89 - protein, 30 aa, Homo sapiens
ISENLKEKKTDAKQQVSGWTPAHVRKQLAI

SEQ ID NO: 90 - protein, 17 aa, Homo sapiens
ERIAPVIGLKCVLALAF

SEQ ID NO: 91 - protein, 18 aa, Homo sapiens
DTSFEDLSKPKRKLADGR

SEQ ID NO: 92 - protein, 23 aa, Homo sapiens
KKLIPNPNKIRKPPKSKKATPKQ

SEQ ID NO: 93 - protein, 27 aa, Homo sapiens
ILKALSGMCNIDTGLTFAAVHCLSGKR

SEQ ID NO: 94 - protein, 23 aa, Homo sapiens
TGIIISDLTMEMNRFRLIGPLSH

SEQ ID NO: 95 - protein, 19 aa, Homo sapiens
QLLLEGVPVECTHSFIWNQ

SEQ ID NO: 96 - protein, 19 aa, Homo sapiens
WHYCGPQESKHSDPFRSKI

SEQ ID NO: 97 - protein, 23 aa, Homo sapiens
SDGPAGEEPVAGQEALTLGLWSG

SEQ ID NO: 98 - protein, 15 aa, Artificial Sequence
  Description of Artificial Sequence: Synthetic peptide
IGDGTRDPCLPYSWI

SEQ ID NO: 99 - protein, 20 aa, Homo sapiens
AFATASMAQPATRAIVFSGC

SEQ ID NO: 100 - protein, 30 aa, Artificial Sequence
  Description of Artificial Sequence: Synthetic polypeptide
TASMAQPATRAIVFSAASLSVLKNVPGLAI

SEQ ID NO: 101 - protein, 26 aa, Artificial Sequence
  Description of Artificial Sequence: Synthetic peptide
EPGVADEDQTAAASLSVLKNVPGLAI

SEQ ID NO: 102 - protein, 15 aa, Artificial Sequence
  Description of Artificial Sequence: Synthetic peptide
DTSFEDLSKPKRKLA

SEQ ID NO: 103 - protein, 23 aa, Artificial Sequence
  Description of Artificial Sequence: Synthetic peptide
TGIIISDLTMEMNRFRLIGPLSH

SEQ ID NO: 104 - protein, 30 aa, Artificial Sequence
  Description of Artificial Sequence: Synthetic polypeptide
DTSFEDLSKPKRKLATGIIISDLTMEMNRF

SEQ ID NO: 105 - protein, 7 aa, Homo sapiens
ATASMAQ

SEQ ID NO: 106 - protein, 14 aa, Homo sapiens
QVSGWTPAHVRKQL

SEQ ID NO: 107 - protein, 10 aa, Homo sapiens
EPGVADEDQT

SEQ ID NO: 108 - protein, 12 aa, Homo sapiens
TQGQTPGEPAAS

SEQ ID NO: 109 - protein, 16 aa, Homo sapiens
LAILLSKDALDPRQPG

SEQ ID NO: 110 - protein, 11 aa, Homo sapiens
EPGVADEDQTA

SEQ ID NO: 111 - protein, 478 aa, Artificial Sequence
  Description of Artificial Sequence: Synthetic polypeptide
  MOD_RES (1)..(150): Any amino acid and this region may encompass 0-50, 0-100 or 0-150 residues, wherein some positions may be absent
  MOD_RES (163)..(312): Any amino acid and this region may encompass 0-50, 0-100 or 0-150 residues, wherein some positions may be absent
  MOD_RES (329)..(478): Any amino acid and this region may encompass 0-50, 0-100 or 0-150 residues, wherein some positions may be absent
XXXXXXXXXXXXXXXXXXXXXXXXXXXXXXXXXXXXXXXXXXXXXXXXXXXXXXXXXXXXXXXXXXXXXXXXXXXXXXXXXXXXXXXXXXXXXXXXXXXXXXXXXXXXXXXXXXXXXXXXXXXXXXXXXXXXXXXXXXXXXXXXXXXXXXATASMAQPATRAXXXXXXXXXXXXXXXXXXXXXXXXXXXXXXXXXXXXXXXXXXXXXXXXXXXXXXXXXXXXXXXXXXXXXXXXXXXXXXXXXXXXXXXXXXXXXXXXXXXXXXXXXXXXXXXXXXXXXXXXXXXXXXXXXXXXXXXXXXXXXXXXXXXXXXKNVPGLAILLSKDALDXXXXXXXXXXXXXXXXXXXXXXXXXXXXXXXXXXXXXXXXXXXXXXXXXXXXXXXXXXXXXXXXXXXXXXXXXXXXXXXXXXXXXXXXXXXXXXXXXXXXXXXXXXXXXXXXXXXXXXXXXXXXXXXXXXXXXXXXXXXXXXXXXXXXXX

SEQ ID NO: 112 - protein, 476 aa, Artificial Sequence
  Description of Artificial Sequence: Synthetic polypeptide
  MOD_RES (1)..(150): Any amino acid and this region may encompass 0-50, 0-100 or 0-150 residues, wherein some positions may be absent
  MOD_RES (163)..(312): Any amino acid and this region may encompass 0-50, 0-100 or 0-150 residues, wherein some positions may be absent
  MOD_RES (327)..(476): Any amino acid and this region may encompass 0-50, 0-100 or 0-150 residues, wherein some positions may be absent
XXXXXXXXXXXXXXXXXXXXXXXXXXXXXXXXXXXXXXXXXXXXXXXXXXXXXXXXXXXXXXXXXXXXXXXXXXXXXXXXXXXXXXXXXXXXXXXXXXXXXXXXXXXXXXXXXXXXXXXXXXXXXXXXXXXXXXXXXXXXXXXXXXXXXXATASMAQPATRAXXXXXXXXXXXXXXXXXXXXXXXXXXXXXXXXXXXXXXXXXXXXXXXXXXXXXXXXXXXXXXXXXXXXXXXXXXXXXXXXXXXXXXXXXXXXXXXXXXXXXXXXXXXXXXXXXXXXXXXXXXXXXXXXXXXXXXXXXXXXXXXXXXXXXXPYIIRWSALESEDMXXXXXXXXXXXXXXXXXXXXXXXXXXXXXXXXXXXXXXXXXXXXXXXXXXXXXXXXXXXXXXXXXXXXXXXXXXXXXXXXXXXXXXXXXXXXXXXXXXXXXXXXXXXXXXXXXXXXXXXXXXXXXXXXXXXXXXXXXXXXXXXXXXXXXX

SEQ ID NO: 113 - protein, 6 aa, Artificial Sequence
  Description of Artificial Sequence: Synthetic 6xHis tag
HHHHHH